European Patent Application EP 4 744 680 A1, published May 20, 2026. Title: Targeted Chemical Drug, Method for Its Preparation, Pharmaceutical Composition, and Uses of the Targeted Chemical Drug. Applicant: BAI YAO ZHI DA (BEIJING) NANOBIO TECHNOLOGY CO., LTD. The sequence listing filed with the application follows.

SEQUENCE LISTING (328 sequences)

SEQ ID NO: 1 - DNA, 12 bp, synthetic construct
  source 1..12: mol_type = other DNA; note = sequence a
acgagcgttccg

SEQ ID NO: 2 - DNA, 10 bp, synthetic construct
  source 1..10: mol_type = other DNA; note = sequence b
cggttcgccg

SEQ ID NO: 3 - DNA, 13 bp, synthetic construct
  source 1..13: mol_type = other DNA; note = sequence c
cggccatagccgt

SEQ ID NO: 4 - RNA, 12 nt, synthetic construct
  source 1..12: mol_type = other RNA; note = sequence a
acgagcgttccg

SEQ ID NO: 5 - RNA, 10 nt, synthetic construct
  source 1..10: mol_type = other RNA; note = sequence b
cggttcgccg

SEQ ID NO: 6 - RNA, 13 nt, synthetic construct
  source 1..13: mol_type = other RNA; note = sequence c
cggccatagccgt

SEQ ID NO: 7 - DNA, 26 bp, synthetic construct
  source 1..26: mol_type = other DNA; note = a-sequence of the 1st set of sequences
gcggcgcccacgagcgttccgggagc

SEQ ID NO: 8 - DNA, 24 bp, synthetic construct
  source 1..24: mol_type = other DNA; note = b-sequence of the 1st set of sequences
gctcccggttcgccgccagccgcc

SEQ ID NO: 9 - DNA, 31 bp, synthetic construct
  source 1..31: mol_type = other DNA; note = c-sequence of the 1st set of sequences
ggcggcaggcggccatagccgtgggcgccgc

SEQ ID NO: 10 - DNA, 31 bp, synthetic construct
  source 1..31: mol_type = other DNA; note = a-sequence of the 2nd set of sequences
gcggcgcccacgagcgttccgggagaggagc

SEQ ID NO: 11 - DNA, 29 bp, synthetic construct
  source 1..29: mol_type = other DNA; note = b-sequence of the 2nd set of sequences
gctcctctcccggttcgccgcgagccgcg

SEQ ID NO: 12 - DNA, 31 bp, synthetic construct
  source 1..31: mol_type = other DNA; note = c-sequence of the 2nd set of sequences
cgcggctcgcggccatagccgtgggcgccgc

SEQ ID NO: 13 - DNA, 30 bp, synthetic construct
  source 1..30: mol_type = other DNA; note = b-sequence of the 3rd set of sequences
gctcctctcccggttcgccgccagccgcgg

SEQ ID NO: 14 - DNA, 31 bp, synthetic construct
  source 1..31: mol_type = other DNA; note = c-sequence of the 3rd set of sequences
ggcggctggcggccatagccgtgggcgccgc

SEQ ID NO: 15 - DNA, 30 bp, synthetic construct
  source 1..30: mol_type = other DNA; note = a-sequence of the 4th set of sequences
gcggcgcccacgagcgttccgggagaggcc

SEQ ID NO: 16 - DNA, 28 bp, synthetic construct
  source 1..28: mol_type = other DNA; note = b-sequence of the 4th set of sequences
ggcctctcccggttcgccgccagccgcc

SEQ ID NO: 17 - RNA, 30 nt, synthetic construct
  source 1..30: mol_type = other RNA; note = a-sequence of the 5th set of sequences
gcggcgcccacgagcgttccgggagaggcc

SEQ ID NO: 18 - RNA, 28 nt, synthetic construct
  source 1..28: mol_type = other RNA; note = b-sequence of the 5th set of sequences
ggcctctcccggttcgccgccagccgcc

SEQ ID NO: 19 - RNA, 31 nt, synthetic construct
  source 1..31: mol_type = other RNA; note = c-sequence of the 5th set of sequences
ggcggctggcggccatagccgtgggcgccgc

SEQ ID NO: 20 - DNA, 33 bp, synthetic construct
  source 1..33: mol_type = other DNA; note = a-sequence of the 6th set of sequences
gcggcgcccacgagcgttccgggagaggaggcc

SEQ ID NO: 21 - DNA, 31 bp, synthetic construct
  source 1..31: mol_type = other DNA; note = b-sequence of the 6th set of sequences
ggcctcctctcccggttcgccgccagccgcc

SEQ ID NO: 22 - DNA, 29 bp, synthetic construct
  source 1..29: mol_type = other DNA; note = b-sequence of the 7th set of sequences
gctcctctcccggttcgccgccagccgcc

SEQ ID NO: 23 - DNA, 30 bp, synthetic construct
  source 1..30: mol_type = other DNA; note = a-sequence of the 8th set of sequences
gcgacgcccacgagcgttccgggagaggag

SEQ ID NO: 24 - DNA, 28 bp, synthetic construct
  source 1..28: mol_type = other DNA; note = b-sequence of the 8th set of sequences
ctcctctcccggttcgccgcgagccgcg

SEQ ID NO: 25 - DNA, 31 bp, synthetic construct
  source 1..31: mol_type = other DNA; note = c-sequence of the 8th set of sequences
cgcggcacgcggccatagccgtgggcgtcgc

SEQ ID NO: 26 - DNA, 31 bp, synthetic construct
  source 1..31: mol_type = other DNA; note = a-sequence of the 9th set of sequences
gcgacgcccacgagcgttccgggagaggagc

SEQ ID NO: 27 - DNA, 31 bp, synthetic construct
  source 1..31: mol_type = other DNA; note = c-sequence of the 9th set of sequences
cgcggctcgcggccatagccgtgggcgtcgc

SEQ ID NO: 28 - DNA, 26 bp, synthetic construct
  source 1..26: mol_type = other DNA; note = a-sequence of the 10th set of sequences
gacgcccacgagcgttccgggagagg

SEQ ID NO: 29 - DNA, 24 bp, synthetic construct
  source 1..24: mol_type = other DNA; note = b-sequence of the 10th set of sequences
cctctcccggttcgccgcgagcct

SEQ ID NO: 30 - DNA, 40 bp, synthetic construct
  source 1..40: mol_type = other DNA; note = c-sequence of the 10th set of sequences
ggctcgcggccatagccgtgggcgtctgctgctgctgctg

SEQ ID NO: 31 - DNA, 21 bp, synthetic construct
  source 1..21: mol_type = other DNA; note = a-sequence of the 11th set of sequences
gcccacgagcgttccgggaga

SEQ ID NO: 32 - DNA, 24 bp, synthetic construct
  source 1..24: mol_type = other DNA; note = b-sequence of the 11th set of sequences
tctcccggttcgccgccagccgcc

SEQ ID NO: 33 - DNA, 26 bp, synthetic construct
  source 1..26: mol_type = other DNA; note = c-sequence of the 11th set of sequences
ggcggctggcggccatagccgtgggc

SEQ ID NO: 34 - RNA, 21 nt, synthetic construct
  source 1..21: mol_type = other RNA; note = sense strand of ASAP1
tgatattatggaagcaaattt

SEQ ID NO: 35 - RNA, 21 nt, synthetic construct
  source 1..21: mol_type = other RNA; note = antisense strand of ASAP1
atttgcttccataatatcatt

SEQ ID NO: 36 - RNA, 21 nt, synthetic construct
  source 1..21: mol_type = other RNA; note = sense strand of ASAP1
ttaggtttggggttggatctt

SEQ ID NO: 37 - RNA, 21 nt, synthetic construct
  source 1..21: mol_type = other RNA; note = antisense strand of ASAP1
gatccaaccccaaacctaatt

SEQ ID NO: 38 - RNA, 21 nt, synthetic construct
  source 1..21: mol_type = other RNA; note = sense strand of ATAD2
aatcctacaacttcgacgctt

SEQ ID NO: 39 - RNA, 21 nt, synthetic construct
  source 1..21: mol_type = other RNA; note = antisense strand of ATAD2
gcgtcgaagttgtaggatttt

SEQ ID NO: 40 - RNA, 21 nt, synthetic construct
  source 1..21: mol_type = other RNA; note = sense strand of CD24
tgtttacattgttgaggtatt

SEQ ID NO: 41 - RNA, 21 nt, synthetic construct
  source 1..21: mol_type = other RNA; note = antisense strand of CD24
tacctcaacaatgtaaacttt

SEQ ID NO: 42 - DNA, 21 bp, synthetic construct
  misc_feature 1..19: note = RNA
  source 1..21: mol_type = other DNA
  misc_feature 20..21: note = DNA
ggtgattacccagagatattt

SEQ ID NO: 43 - DNA, 21 bp, synthetic construct
  misc_feature 1..19: note = RNA
  source 1..21: mol_type = other DNA
  misc_feature 20..21: note = DNA
atatctctgggtaatcacctt

SEQ ID NO: 44 - RNA, 21 nt, synthetic construct
  source 1..21: mol_type = other RNA; note = sense strand of CD47
tggtgaaagaggtcattcctt

SEQ ID NO: 45 - RNA, 21 nt, synthetic construct
  source 1..21: mol_type = other RNA; note = antisense strand of CD47
ggaatgacctctttcaccatt

SEQ ID NO: 46 - DNA, 21 bp, synthetic construct
  misc_feature 1..19: note = RNA
  source 1..21: mol_type = other DNA
  misc_feature 20..21: note = DNA
ggaatgacctctttcaccatt

SEQ ID NO: 47 - DNA, 21 bp, synthetic construct
  misc_feature 1..19: note = RNA
  source 1..21: mol_type = other DNA
  misc_feature 20..21: note = DNA
tggtgaaagaggtcattcctt

SEQ ID NO: 48 - RNA, 21 nt, synthetic construct
  source 1..21: mol_type = other RNA; note = sense strand of CD47
ggtgattacccagagatattt

SEQ ID NO: 49 - RNA, 21 nt, synthetic construct
  source 1..21: mol_type = other RNA; note = antisense strand of CD47
atatctctgggtaatcacctt

SEQ ID NO: 50 - RNA, 21 nt, synthetic construct
  source 1..21: mol_type = other RNA; note = sense strand of EGFR
ggctggttatgtcctcatttt

SEQ ID NO: 51 - RNA, 21 nt, synthetic construct
  source 1..21: mol_type = other RNA; note = antisense strand of EGFR
aatgaggacataaccagcctt

SEQ ID NO: 52 - RNA, 21 nt, synthetic construct
  source 1..21: mol_type = other RNA; note = sense strand of EGFR
ttagataagactgctaaggtt

SEQ ID NO: 53 - RNA, 21 nt, synthetic construct
  source 1..21: mol_type = other RNA; note = antisense strand of EGFR
ttagataagactgctaaggtt

SEQ ID NO: 54 - RNA, 23 nt, synthetic construct
  source 1..23: mol_type = other RNA; note = sense strand of EGFR
tgccttagcagtcttatctaatt

SEQ ID NO: 55 - RNA, 23 nt, synthetic construct
  source 1..23: mol_type = other RNA; note = antisense strand of EGFR
ttagataagactgctaaggcatt

SEQ ID NO: 56 - RNA, 21 nt, synthetic construct
  source 1..21: mol_type = other RNA; note = sense strand of HBV
ggacttctctcaattttcttt

SEQ ID NO: 57 - RNA, 21 nt, synthetic construct
  source 1..21: mol_type = other RNA; note = antisense strand of HBV
agaaaattgagagaagtcctt

SEQ ID NO: 58 - RNA, 21 nt, synthetic construct
  source 1..21: mol_type = other RNA; note = sense strand of HSP
cgcagaacaccgtgttcgatt

SEQ ID NO: 59 - RNA, 21 nt, synthetic construct
  source 1..21: mol_type = other RNA; note = antisense strand of HSP
tcgaacacggtgttctgcgtt

SEQ ID NO: 60 - RNA, 21 nt, synthetic construct
  source 1..21: mol_type = other RNA; note = sense strand of HS70
ggccaacaagatcaccatctt

SEQ ID NO: 61 - RNA, 21 nt, synthetic construct
  source 1..21: mol_type = other RNA; note = antisense strand of HS70
gatggtgatcttgttggcctt

SEQ ID NO: 62 - RNA, 21 nt, synthetic construct
  source 1..21: mol_type = other RNA; note = sense strand of PD-L1
ccagcacactgagaatcaatt

SEQ ID NO: 63 - RNA, 21 nt, synthetic construct
  source 1..21: mol_type = other RNA; note = antisense strand of PD-L1
ttgattctcagtgtgctggtt

SEQ ID NO: 64 - DNA, 21 bp, synthetic construct
  misc_feature 1..19: note = RNA
  source 1..21: mol_type = other DNA
  misc_feature 20..21: note = DNA
agacgtaagcagtgttgaatt

SEQ ID NO: 65 - DNA, 21 bp, synthetic construct
  misc_feature 1..19: note = RNA
  source 1..21: mol_type = other DNA
  misc_feature 20..21: note = DNA
ttcaacactgcttacgtcttt

SEQ ID NO: 66 - DNA, 21 bp, synthetic construct
  misc_feature 1..19: note = RNA
  source 1..21: mol_type = other DNA
  misc_structure 20..21: note = DNA
gaggaaggtatcaacaaattt

SEQ ID NO: 67 - DNA, 21 bp, synthetic construct
  misc_feature 1..19: note = RNA
  source 1..21: mol_type = other DNA
  misc_feature 20..21: note = DNA
atttgttgataccttcctctt

SEQ ID NO: 68 - DNA, 51 bp, synthetic construct
  source 1..51: mol_type = other DNA; note = C sequence
ccctcctacatagggtttttggcggctggcggccatagccgtgggcgccgc

SEQ ID NO: 69 - DNA, 45 bp, synthetic construct
  source 1..45: mol_type = other DNA; note = PD-L1
acgggccacatcaactcattgatagacaatgcgtccactgcccgt

SEQ ID NO: 70 - RNA, 23 nt, synthetic construct
  source 1..23: mol_type = other RNA; note = sense strand of Survivin
gcaggttccttatctgtcacatt

SEQ ID NO: 71 - RNA, 25 nt, synthetic construct
  source 1..25: mol_type = other RNA; note = antisense strand of Survivin
tgtgacagataaggaacctgcagtt

SEQ ID NO: 72 - RNA, 23 nt, synthetic construct
  source 1..23: mol_type = other RNA; note = sense strand of Survivin
ggaattggaaggctgggaacctt

SEQ ID NO: 73 - RNA, 23 nt, synthetic construct
  source 1..23: mol_type = other RNA; note = antisense strand of Survivin
ggttcccagccttccaattcctt

SEQ ID NO: 74 - DNA, 22 bp, synthetic construct
  misc_feature 1..20: note = RNA
  source 1..22: mol_type = other DNA
  misc_feature 21..22: note = DNA
tgcaggttccttatctgtcatt

SEQ ID NO: 75 - DNA, 21 bp, synthetic construct
  misc_feature 1..19: note = RNA
  source 1..21: mol_type = other DNA
  misc_feature 20..21: note = DNA
tgacagataaggaacctgctt

SEQ ID NO: 76 - RNA, 25 nt, synthetic construct
  source 1..25: mol_type = other RNA; note = sense strand of Survivin
ctgcaggttccttatctgtcacatt

SEQ ID NO: 77 - RNA, 25 nt, synthetic construct
  source 1..25: mol_type = other RNA; note = antisense strand of Survivin
tgtgacagataaggaacctgcagtt

SEQ ID NO: 78 - RNA, 25 nt, synthetic construct
  source 1..25: mol_type = other RNA; note = sense strand of EGFR
tgccttagcagtcttatctaatttt

SEQ ID NO: 79 - RNA, 25 nt, synthetic construct
  source 1..25: mol_type = other RNA; note = antisense strand of EGFR
aattagataagactgctaaggcatt

SEQ ID NO: 80 - RNA, 21 nt, synthetic construct
  source 1..21: mol_type = other RNA; note = sense strand of TAP
gctgcacacggttcagaattt

SEQ ID NO: 81 - RNA, 21 nt, synthetic construct
  source 1..21: mol_type = other RNA; note = antisense strand of TAP
attctgaaccgtgtgcagctt

SEQ ID NO: 82 - RNA, 21 nt, synthetic construct
  source 1..21: mol_type = other RNA; note = sense strand of TAP
caggatgagttacttgaaatt

SEQ ID NO: 83 - RNA, 21 nt, synthetic construct
  source 1..21: mol_type = other RNA; note = antisense strand of TAP
tttcaagtaactcatcctgtt

SEQ ID NO: 84 - RNA, 25 nt, synthetic construct
  source 1..25: mol_type = other RNA; note = sense strand of VEGF-C
cagcaagacgttgtttgaaattatt

SEQ ID NO: 85 - RNA, 25 nt, synthetic construct
  source 1..25: mol_type = other RNA; note = antisense strand of VEGF-C
taatttcaaacaacgtcttgctgtt

SEQ ID NO: 86 - DNA, 21 bp, synthetic construct
  misc_feature 1..19: note = RNA
  source 1..21: mol_type = other DNA
  misc_feature 20..21: note = DNA
gtgctcaggactgatgaaatt

SEQ ID NO: 87 - DNA, 21 bp, synthetic construct
  misc_feature 1..19: note = RNA
  source 1..21: mol_type = other DNA
  misc_feature 20..21: note = DNA
tttcatcagtcctgagcactt

SEQ ID NO: 88 - RNA, 21 nt, synthetic construct
  source 1..21: mol_type = other RNA; note = sense strand of TGF-beta1
gtcaactgtggagcaacactt

SEQ ID NO: 89 - RNA, 21 nt, synthetic construct
  source 1..21: mol_type = other RNA; note = antisense strand of TGF-beta1
gtgttgctccacagttgactt

SEQ ID NO: 90 - DNA, 21 bp, synthetic construct
  misc_feature 1..19: note = RNA
  source 1..21: mol_type = other DNA
  misc_feature 20..21: note = DNA
gcaacaacgccatctatgatt

SEQ ID NO: 91 - DNA, 21 bp, synthetic construct
  misc_feature 1..19: note = RNA
  source 1..21: mol_type = other DNA
  misc_feature 20..21: note = DNA
tcatagatggcgttgttgctt

SEQ ID NO: 92 - RNA, 23 nt, synthetic construct
  source 1..23: mol_type = other RNA; note = sense strand of VEGF-C
gcaagacgttgtttgaaattatt

SEQ ID NO: 93 - RNA, 23 nt, synthetic construct
  source 1..23: mol_type = other RNA; note = antisense strand of VEGF-C
taatttcaaacaacgtcttgctt

SEQ ID NO: 94 - RNA, 21 nt, synthetic construct
  source 1..21: mol_type = other RNA; note = sense strand of VEGF-C
caggatggtaaagactacatt

SEQ ID NO: 95 - RNA, 21 nt, synthetic construct
  source 1..21: mol_type = other RNA; note = antisense strand of VEGF-C
tgtagtctttaccatcctgtt

SEQ ID NO: 96 - DNA, 23 bp, synthetic construct
  source 1..23: mol_type = other DNA; note = A-miR21
gtcaacatcagtctgataagcta

SEQ ID NO: 97 - RNA, 23 nt, synthetic construct
  source 1..23: mol_type = other RNA; note = A-miR21
gtcaacatcagtctgataagcta

SEQ ID NO: 98 - DNA, 22 bp, synthetic construct
  source 1..22: mol_type = other DNA; note = A-miR21
tcaacatcagtctgataagcta

SEQ ID NO: 99 - DNA, 23 bp, synthetic construct
  source 1..23: mol_type = other DNA; note = A-miR-30c
gctgagagtgtaggatgtttaca

SEQ ID NO: 100 - DNA, 22 bp, synthetic construct
  source 1..22: mol_type = other DNA; note = AmiR-1306
catcaccaccagagccaacgtc

SEQ ID NO: 101 - DNA, 45 bp, synthetic construct
  source 1..45: mol_type = other DNA; note = A1
ggttgcatgccgtggggaggggggtgggttttatagcgtactcag

SEQ ID NO: 102 - DNA, 15 bp, synthetic construct
  source 1..15: mol_type = other DNA; note = A15
ccctcctacataggg

SEQ ID NO: 103 - DNA, 26 bp, synthetic construct
  source 1..26: mol_type = other DNA; note = AS1411
ggtggtggtggttgtggtggtggtgg

SEQ ID NO: 104 - DNA, 72 bp, synthetic construct
  source 1..72: mol_type = other DNA; note = AFP
ggcaggaagacaaacaagcttggcggcgggaaggtgtttaaattcccgggtctgcgtggtctgtggtgctgt

SEQ ID NO: 105 - DNA, 25 bp, synthetic construct
  source 1..25: mol_type = other DNA; note = AFP
acctggggagtattggggaggaagg

SEQ ID NO: 106 - DNA, 25 bp, synthetic construct
  source 1..25: mol_type = other DNA; note = ATP
acctggggagtattggggaggaagg

SEQ ID NO: 107 - DNA, 27 bp, synthetic construct
  source 1..27: mol_type = other DNA; note = ATP
gggaggacgatgcggaggaagggtagg

SEQ ID NO: 108 - DNA, 45 bp, synthetic construct
  source 1..45: mol_type = other DNA; note = Act-12c
cggggaaagtcacggggggtttcagatgttctgatcggtgtggag

SEQ ID NO: 109 - DNA, 15 bp, synthetic construct
  source 1..15: mol_type = other DNA; note = A18
ccagatagtccctgg

SEQ ID NO: 110 - DNA, 24 bp, synthetic construct
  source 1..24: mol_type = other DNA; note = BAF7-1
gataacgggcacgaattcggagtg

SEQ ID NO: 111 - DNA, 50 bp, synthetic construct
  source 1..50: mol_type = other DNA; note = C-Met-SL1
atcaggctggatggtagctcggtcggggtgggtgggttggcaagtctgat

SEQ ID NO: 112 - DNA, 40 bp, synthetic construct
  source 1..40: mol_type = other DNA; note = CH6
agtctgttggaccgaatcccgtggacgcaccctttggacg

SEQ ID NO: 113 - DNA, 36 bp, synthetic construct
  source 1..36: mol_type = other DNA; note = CA2
cccacgtctgcgcttagctcctgggcctggatgggc

SEQ ID NO: 114 - DNA, 35 bp, synthetic construct
  source 1..35: mol_type = other DNA; note = C12
gtggattgttgtgttctgttggtttttgtgttgtc

SEQ ID NO: 115 - DNA, 40 bp, synthetic construct
  source 1..40: mol_type = other DNA; note = CRAC Orail
ccagtagccataccggtttgtggatggggtgtatgcgagt

SEQ ID NO: 116 - DNA, 40 bp, synthetic construct
  source 1..40: mol_type = other DNA; note = CEA
ctaggatccccactcaccatctctcagcttgcttcctagc

SEQ ID NO: 117 - DNA, 18 bp, synthetic construct
  source 1..18: mol_type = other DNA; note = CEA-18
ttaacttattcgaccata

SEQ ID NO: 118 - DNA, 71 bp, synthetic construct
  source 1..71: mol_type = other DNA; note = CEA-T84
tcgcgcgagtcgtctggggaaccatcgagttacaccgaccttctatgtgcggccccccgcatcgtcctccc

SEQ ID NO: 119 - DNA, 78 bp, synthetic construct
  source 1..78: mol_type = other DNA; note = CSC1
accttggctgtcgtgttgtaggtggtttgctgcggtgggctcaagaagaaagcgcaaagaggtcagtggtcagagcgt

SEQ ID NO: 120 - DNA, 78 bp, synthetic construct
  source 1..78: mol_type = other DNA; note = CSC13
accttggctgtcgtgttgtggggtgtcgtatctttcgtgtcttattattttctaggtggaggtcagtggtcagagcgt

SEQ ID NO: 121 - DNA, 25 bp, synthetic construct
  source 1..25: mol_type = other DNA; note = CD40
ccaacgagtaggcgatagcgcgtgg

SEQ ID NO: 122 - DNA, 50 bp, synthetic construct
  source 1..50: mol_type = other DNA; note = CD40
agagacgatgcggccaacgagtaggcgatagcgcgtggcagagcgtcgct

SEQ ID NO: 123 - DNA, 34 bp, synthetic construct
  source 1..34: mol_type = other DNA; note = CD16a
ccactgcgggggtctatacgtgaggaagaagtgg

SEQ ID NO: 124 - DNA, 61 bp, synthetic construct
  source 1..61: mol_type = other DNA; note = CD19
tgcgtgtgtagtgtgtgtcgtttctcctttttttggttgctgctcttagggatttgggcgg

SEQ ID NO: 125 - DNA, 59 bp, synthetic construct
  source 1..59: mol_type = other DNA; note = CD19
tgcgtgtgtagtgtgtctgttctcctttttttggttgctgctcttagggatttgggcgg

SEQ ID NO: 126 - DNA, 87 bp, synthetic construct
  source 1..87: mol_type = other DNA; note = CD3-4
tctcggacgcgtgtggtcggccgagtggcccacggtagaagggttagaactgctggttggtgaatctcgctgcctggccctagagtg

SEQ ID NO: 127 - DNA, 30 bp, synthetic construct
  source 1..30: mol_type = other DNA; note = CD44
ccaaggcctgcaagggaaccaaggacacag

SEQ ID NO: 128 - DNA, 30 bp, synthetic construct; identical to SEQ ID NO: 127
  source 1..30: mol_type = other DNA; note = CD44

SEQ ID NO: 129 - DNA, 35 bp, synthetic construct; identical to SEQ ID NO: 114
  source 1..35: mol_type = other DNA; note = CD12(HDLBP)

SEQ ID NO: 130 - DNA, 59 bp, synthetic construct
  source 1..59: mol_type = other DNA; note = CD20
tgcgtgtgtagtgtgtctgttttttatcttcttttatctactcttagggatttgggcgg

SEQ ID NO: 131 - DNA, 40 bp, synthetic construct
  source 1..40: mol_type = other DNA; note = CD24
tatgtgggtgggtgggcggttatgctgagtcagccttgct

SEQ ID NO: 132 - DNA, 76 bp, synthetic construct
  source 1..76: mol_type = other DNA; note = CD24
atccagagtgacgcagcatatgtgggtgggtgggcggttatgctgagtcagccttgcttggacacggtggcttagt

SEQ ID NO: 133 - DNA, 57 bp, synthetic construct
  source 1..57: mol_type = other DNA; note = CD33
taccagtgcgatgctcagcacgcttataggggctggacaaaattctacccagccttt

SEQ ID NO: 134 - DNA, 32 bp, synthetic construct
  source 1..32: mol_type = other DNA; note = CD38
tacgtgaatctcgtacgatactctgtaagcgt

SEQ ID NO: 135 - DNA, 45 bp, synthetic construct
  source 1..45: mol_type = other DNA; note = CD105
gatcagttttccatgccagttggtattccgcgacagtttgatctc

SEQ ID NO: 136 - DNA, 35 bp, synthetic construct
  source 1..35: mol_type = other DNA; note = CD117
ggggccggggcaaggggggggtaccgtggtaggac

SEQ ID NO: 137 - DNA, 32 bp, synthetic construct
  source 1..32: mol_type = other DNA; note = CD63
caccccacctcgctcccgtgacactaatgcta

SEQ ID NO: 138 - DNA, 66 bp, synthetic construct
  source 1..66: mol_type = other DNA; note = CD123
tgcgtgtgtagtgtgtctgggctacatcgatgagctgcctagggtccctcttagggatttgggcgg

SEQ ID NO: 139 - DNA, 39 bp, synthetic construct
  source 1..39: mol_type = other DNA; note = EGFR
gccttagtaacgtgctttgatgtcgattcgacaggaggc

SEQ ID NO: 140 - DNA, 48 bp, synthetic construct
  source 1..48: mol_type = other DNA; note = EpCAM
cactacagaggttgcgtctgtcccacgttgtcatggggggttggcctg

SEQ ID NO: 141 - DNA, 31 bp, synthetic construct
  source 1..31: mol_type = other DNA; note = EpCAM
gacaaacgggggaagatttgacgtcgacgac

SEQ ID NO: 142 - DNA, 47 bp, synthetic construct
  source 1..47: mol_type = other DNA; note = EcR
gcaggtccactgcgggggtctatacgtgaggaagaagtgggcaggtc

SEQ ID NO: 143 - DNA, 21 bp, synthetic construct
  source 1..21: mol_type = other DNA; note = FAP
tgggggttgaggctaagccga

SEQ ID NO: 144 - DNA, 31 bp, synthetic construct
  source 1..31: mol_type = other DNA; note = anti-FAP
ccgctcgagctagtctgacaaagagaaacac

SEQ ID NO: 145 - DNA, 21 bp, synthetic construct
  source 1..21: mol_type = other DNA; note = GPC-1
aacggagtgtggctaactcga

SEQ ID NO: 146 - DNA, 54 bp, synthetic construct
  source 1..54: mol_type = other DNA; note = H2
gggccgtcgaacacgagcatggtgcgtggacctaggatgacctgagtactgtcc

SEQ ID NO: 147 - DNA, 20 bp, synthetic construct
  source 1..20: mol_type = other DNA; note = GSK836
gcagaggtgaagcgaagtcg

SEQ ID NO: 148 - DNA, 37 bp, synthetic construct
  source 1..37: mol_type = other DNA; note = GPC3(APS63-1)
taacgctgaccttagctgcatggctttacatgttcca

SEQ ID NO: 149 - DNA, 34 bp, synthetic construct
  source 1..34: mol_type = other DNA; note = Her2
agccgcgaggggagggatagggtagggcgcggct

SEQ ID NO: 150 - DNA, 81 bp, synthetic construct
  source 1..81: mol_type = other DNA; note = Her2
gggagctcagaataaacgctcaaagggtcaagctgattacactttgtccactattgggtccttcgacatgaggcccggatc

SEQ ID NO: 151 - DNA, 81 bp, synthetic construct
  source 1..81: mol_type = other DNA; note = Her3
gggagctcagaataaacgctcaaggctaacagcacgcaacgggggggagtaatcgtgtctgttcgacatgaggcccggatc

SEQ ID NO: 152 - DNA, 23 bp, synthetic construct
  source 1..23: mol_type = other DNA; note = HMGA2
ggaaaaaattttttaaaaaaccc

SEQ ID NO: 153 - DNA, 40 bp, synthetic construct
  source 1..40: mol_type = other DNA; note = HBsAg
cacagcgaacagcggcggacataatagtgcttactacgac

SEQ ID NO: 154 - DNA, 63 bp, synthetic construct
  source 1..63: mol_type = other DNA; note = IFN-y(B4)
ccgcccaaatccctaagagaagactgtaatgacatcaaaccagacacacacactacacacgca

SEQ ID NO: 155 - RNA, 79 nt, synthetic construct
  source 1..79: mol_type = other RNA; note = IL-4Ra
ggaggacgatgcggaaaaagcaacagggtgctccatgcgcatggaacctgcgcgcagacgactcgctgaggatccgaga

SEQ ID NO: 156 - RNA, 40 nt, synthetic construct
  source 1..40: mol_type = other RNA; note = IL-4Ra
aaaaagcaacagggtgctccatgcgcatggaacctgcgcg

SEQ ID NO: 157 - DNA, 30 bp, synthetic construct
  source 1..30: mol_type = other DNA; note = IL-17
cttggatcaccatagtcgctagtcgaggct

SEQ ID NO: 158 - DNA, 24 bp, synthetic construct
  source 1..24: mol_type = other DNA; note = IL-17
gcggcatcctatcacgcattgacc

SEQ ID NO: 159 - DNA, 60 bp, synthetic construct
  source 1..60: mol_type = other DNA; note = LZH8
atccagagtgacgcagcatattagtacggcttaaccccatggtggacacggtggcttagt

SEQ ID NO: 160 - DNA, 25 bp, synthetic construct
  source 1..25: mol_type = other DNA; note = MUC1
gcagttgatcctttggataccctgg

SEQ ID NO: 161 - DNA, 25 bp, synthetic construct
  source 1..25: mol_type = other DNA; note = MUC1
gaagtgaaaatgacagaacacaaca

SEQ ID NO: 162 - DNA, 88 bp, synthetic construct
  source 1..88: mol_type = other DNA; note = MUC1
aaccgcccaaatctctaagagtcggactgcaacctatgctatcgttgatgtctgtccaagcaacacagacacactacacacacgcaca

SEQ ID NO: 163 - DNA, 19 bp, synthetic construct
  source 1..19: mol_type = other DNA; note = MUC1
aatgacagaacacaacatt

SEQ ID NO: 164 - DNA, 80 bp, synthetic construct
  source 1..80: mol_type = other DNA; note = M5
agcagcacagaggtcagatgcttggttccaccgtactgactgtagtaaaatctgatcactcctatgcgtgctaccgtgaa

SEQ ID NO: 165 - DNA, 80 bp, synthetic construct
  source 1..80: mol_type = other DNA; note = M7
agcagcacagaggtcagatgtagtcggtcttcttgtttgaaactgctaattttgaaaaaacctatgcgtgctaccgtgaa

SEQ ID NO: 166 - DNA, 80 bp, synthetic construct
  source 1..80: mol_type = other DNA; note = M1
agcagcacagaggtcagatgatataaccttaataaataaaatataaattatttaatcttacctatgcgtgctaccgtgaa

SEQ ID NO: 167 - DNA, 40 bp, synthetic construct
  source 1..40: mol_type = other DNA; note = N5
gattgagtagatagtggttctgtacgtagtgaaagagtgg

SEQ ID NO: 168 - DNA, 94 bp, synthetic construct
  source 1..94: mol_type = other DNA; note = N-G-Dua
caagttgctcgtcgcgatacgtttggttggtgtggttggcagtatcgcaggtccaagttgctcgtcgcgatacaacggagtgtggctaactcga

SEQ ID NO: 169 - DNA, 46 bp, synthetic construct
  source 1..46: mol_type = other DNA; note = NKG2D(20-N-15)
caagttgctcgtcgcgatacgtttggttggtgtggttggcagtatc

SEQ ID NO: 170 - DNA, 39 bp, synthetic construct
  source 1..39: mol_type = other DNA; note = NSE
tcacacggacctctctctacattaattgcgcatttcgtt

SEQ ID NO: 171 - DNA, 58 bp, synthetic construct
  source 1..58: mol_type = other DNA; note = Np-A15
gctggatgttcatgctggcaaaattccttaggggcaccgttactttgacacatccagc

SEQ ID NO: 172 - DNA, 58 bp, synthetic construct
  source 1..58: mol_type = other DNA; note = Np-A48
gctggatgtcgcttacgacaatattccttaggggcaccgctacattgacacatccagc

SEQ ID NO: 173 - DNA, 58 bp, synthetic construct
  source 1..58: mol_type = other DNA; note = Np-A58
gctggatgtcaccggattgtcggacatcggattgtctgagtcatatgacacatccagc

SEQ ID NO: 174 - DNA, 58 bp, synthetic construct
  source 1..58: mol_type = other DNA; note = Np-A61
gctggatgttgacctttacagatcggattctgtggggcgttaaactgacacatccagc

SEQ ID NO: 175 - DNA, 80 bp, synthetic construct
  source 1..80: mol_type = other DNA; note = OX40
gggaggacgatgcggcagtctgcatcgtaggaatcgccaccgtatactttcccaccagacgactcgctgaggatccgaga

SEQ ID NO: 176 - DNA, 39 bp, synthetic construct
  source 1..39: mol_type = other DNA; note = OX40
  misc_feature 1..27: note = DNA
  misc_feature 28: note = RNA
  misc_structure 29..39: note = DNA
cagtctgcatcgtaggattagccaccgtatctttcccac

SEQ ID NO: 177 - DNA, 25 bp, synthetic construct
  source 1..25: mol_type = other DNA; note = OX40
ccaacgagtaggcgatagcgcgtgg

SEQ ID NO: 178 - DNA, 73 bp, synthetic construct
  source 1..73: mol_type = other DNA; note = B sequence
gccttagtaacgtgctttgatgtcgattcgacaggaggctttttgctcctctcccggttcgccgccagccgcc

SEQ ID NO: 179 - DNA, 39 bp, synthetic construct
  source 1..39: mol_type = other DNA; note = PSMA
gggaggacgatgcggatcagccatgtttacgtcactcct

SEQ ID NO: 180 - DNA, 48 bp, synthetic construct
  source 1..48: mol_type = other DNA; note = PSMA
gcgttttcgcttttgcgttttgggtcatctgcttacgatagcaatgct

SEQ ID NO: 181 - DNA, 33 bp, synthetic construct
  source 1..33: mol_type = other DNA; note = PDGFRbeta
tgtcgtggggcatcgagtaaatgcaattcgaca

SEQ ID NO: 182 - DNA, 35 bp, synthetic construct
  source 1..35: mol_type = other DNA; note = PDGF
caggctacggcacgtagagcatcaccatgatcctg

SEQ ID NO: 183 - DNA, 40 bp, synthetic construct
  source 1..40: mol_type = other DNA; note = PD-L1
aacaacgtataacaatgcccacgtcaccagagtactatgg

SEQ ID NO: 184 - DNA, 33 bp, synthetic construct
  source 1..33: mol_type = other DNA; note = PD-L1
gccccagttatgctttccccctctgtctctttg

SEQ ID NO: 185 - DNA, 31 bp, synthetic construct
  source 1..31: mol_type = other DNA; note = PD-L1
atcgcccgcagcacccatttgtttttttttg

SEQ ID NO: 186 - DNA, 45 bp, synthetic construct
  source 1..45: mol_type = other DNA; note = PD-L1
tgcccgcacatcaactcattgatagacaatgcgtccactcgggca

SEQ ID NO: 187 - DNA, 45 bp, synthetic construct
  source 1..45: mol_type = other DNA; note = PD-L1
tgcccgcacatcaactcattgatagacaatgcgtccactacgggc

SEQ ID NO: 188 - DNA, 45 bp, synthetic construct
  source 1..45: mol_type = other DNA; note = PD-L1
cgggcacacatcaactcattgatagacaatgcgtccactgcccgt

SEQ ID NO: 189 - DNA, 45 bp, synthetic construct
  source 1..45: mol_type = other DNA; note = PD-L1
gttggtcacatcaactcattgatagacaatgcgtccactaccaac

SEQ ID NO: 190 - DNA, 41 bp, synthetic construct
  source 1..41: mol_type = other DNA; note = PD-L1
gggccacatcaactcattgatagacaatgcgtccactgccc

SEQ ID NO: 191 - DNA, 45 bp, synthetic construct
  source 1..45: mol_type = other DNA; note = PD-L1
tggttgcacatcaactcattgatagacaatgcgtccactcaacca

SEQ ID NO: 192 - DNA, 75 bp, synthetic construct
  source 1..75: mol_type = other DNA; note = PD-1
gacgatagcggtgacggcacagacggtacagttcccgtccctgcactacacgtatgccgcttccgtccgtcgctc

SEQ ID NO: 193 - DNA, 75 bp, synthetic construct
  source 1..75: mol_type = other DNA; note = PD-1
gagcgacggacggaagcggcatacgtgtagtgcagggacgggaactgtaccgtctgtgccgtcaccgctatcgtc

SEQ ID NO: 194 - DNA, 70 bp, synthetic construct
  source 1..70: mol_type = other DNA; note = PD-1
ggatcctagacgcattgacccgctgcctctactgaggctgtgtcagtgtgcggctcggactgttgaattc

SEQ ID NO: 195 - DNA, 70 bp, synthetic construct
  source 1..70: mol_type = other DNA; note = PD-1
agcggtgacggcacagacggtacagttcccgtccctgcactacacgtatgccgctgagagagagggaggc

SEQ ID NO: 196 - DNA, 40 bp, synthetic construct
  source 1..40: mol_type = other DNA; note = PD-1
accgacagtgaaggactcagcgaactctcagactcggttc

SEQ ID NO: 197 - DNA, 41 bp, synthetic construct
  source 1..41: mol_type = other DNA; note = PTK-7
atctaactgctgcgccgccgggaaaatactgtacggttaga

SEQ ID NO: 198 - DNA, 47 bp, synthetic construct
  source 1..47: mol_type = other DNA; note = ProGRP-48
catgcggagtagagcgagcccagatagtccctggttatttccttagg

SEQ ID NO: 199 - DNA, 40 bp, synthetic construct
  source 1..40: mol_type = other DNA; note = SF
gatctctctctgccctaagtccgcacccgtgcttccctgt

SEQ ID NO: 200 - DNA, 33 bp, synthetic construct
  source 1..33: mol_type = other DNA; note = PD-L1
tacaggttctggggggtgggtggggaacctgtt

SEQ ID NO: 201 - DNA, 15 bp, synthetic construct
  source 1..15: mol_type = other DNA; note = TBA15
ggttggtgtggttgg

SEQ ID NO: 202 - DNA, 29 bp, synthetic construct
  source 1..29: mol_type = other DNA; note = TBA29
agtccgtggtagggcaggttggggtgact

SEQ ID NO: 203 - DNA, 14 bp, synthetic construct
  source 1..14: mol_type = other DNA; note = TfRA4
gcgtggtaccacgc

SEQ ID NO: 204 - DNA, 14 bp, synthetic construct
  source 1..14: mol_type = other DNA; note = TfRA3
gcgtggtcacacgc

SEQ ID NO: 205 - DNA, 74 bp, synthetic construct
  source 1..74: mol_type = other DNA; note = TfRA3
gcggcgcccacgagcgttcgcgtggtcacacgcgttccgccctcctacatagggcgcatagccgtgggcgccgc

SEQ ID NO: 206 - DNA, 34 bp, synthetic construct
  source 1..34: mol_type = other DNA; note = TTA1
cctgcacttggcttggatttcagaagggagaccc

SEQ ID NO: 207 - DNA, 39 bp, synthetic construct
  source 1..39: mol_type = other DNA; note = TLS9a
agtccattttattcctgaatatttgttaacctcatggac

SEQ ID NO: 208 - DNA, 60 bp, synthetic construct
  source 1..60: mol_type = other DNA; note = TGF-betaII(S58)
acattgctgcgtgatcgcctcacatgggtttgtctggtcgatttggaggtggtgggtggc

SEQ ID NO: 209 - DNA, 33 bp, synthetic construct
  source 1..33: mol_type = other DNA; note = TNF-a
gcggccgataaggtctttccaagcgaacgaaaa

SEQ ID NO: 210 - DNA, 41 bp, synthetic construct
  source 1..41: mol_type = other DNA; note = TNF
gcgccactacaggggagctgccattcgaataggtgggccgc

SEQ ID NO: 211 - DNA, 74 bp, synthetic construct
  source 1..74: mol_type = other DNA; note = T1
cgctcgatagatcgagcttcgctcgatgtggtgttgtgggggcttgtattggtcgatcacgctctagagcactg

SEQ ID NO: 212 - DNA, 25 bp, synthetic construct
  source 1..25: mol_type = other DNA; note = VEGF
tgtgggggtggactgggtgggtacc

SEQ ID NO: 213 - DNA, 25 bp, synthetic construct
  source 1..25: mol_type = other DNA; note = VEGF
tgtgggggtggacgggccgggtaga

SEQ ID NO: 214 - DNA, 25 bp, synthetic construct
  source 1..25: mol_type = other DNA; note = VEGF
ggtgggggtggacgggccgggtaga

SEQ ID NO: 215 - DNA, 95 bp, synthetic construct
  source 1..95: mol_type = other DNA; note = VCAM-1
ataccagcttattcaattggacacggcaaaggggtatagcctaccggaccgtgaacatggaatggtgtgctgcgtggagatagtaagtgcaatct

SEQ ID NO: 216 - DNA, 59 bp, synthetic construct
  source 1..59: mol_type = other DNA; note = VCAM-1
ggacacggcaaaggggtatagcctaccggaccgtgaacatggaatggtgtgctgcgtgg

SEQ ID NO: 217 - DNA, 39 bp, synthetic construct
  source 1..39: mol_type = other DNA; note = VCAM-12d
agggaatcttgcctagggagggagtagcgaaagggctca

SEQ ID NO: 218 - DNA, 40 bp, synthetic construct; identical to SEQ ID NO: 112
  source 1..40: mol_type = other DNA; note = CH6

SEQ ID NO: 219 - DNA, 56 bp, synthetic construct
  source 1..56: mol_type = other DNA; note = PL-45
actcatagggttaggggctgctggccagatactcagatggtagggttactatgagc

SEQ ID NO: 220 - DNA, 40 bp, synthetic construct
  source 1..40: mol_type = other DNA; note = EP66
aacagagggacaaacgggggaagatttgacgtcgacgaca

SEQ ID NO: 221 - DNA, 52 bp, synthetic construct
  source 1..52: mol_type = other DNA; note = AGC
cgacccggcacaaacccagaaccatatacacgatcattcgtctcctgggccg

SEQ ID NO: 222 - DNA, 52 bp, synthetic construct
  source 1..52: mol_type = other DNA; note = Karpas299
atccagatgacgcagcaccaccaccgtacaattttttcattacctactcggc

SEQ ID NO: 223 - DNA, 45 bp, synthetic construct
  source 1..45: mol_type = other DNA; note = SW620
cccatcaatgttacgacccgctagggctgctgtgccatcgggtaa

SEQ ID NO: 224 - DNA, 66 bp, synthetic construct
  source 1..66: mol_type = other DNA; note = MDA-MB-231
agaattcagtcggacagcgaagtagttttccttctaacctaagaacccgcggcagtttaatgtaga

SEQ ID NO: 225 - DNA, 45 bp, synthetic construct
  source 1..45: mol_type = other DNA; note = MCF-7
gcatggggtttcggcgtttcgtctatcttgtttctgttagcgtct

SEQ ID NO: 226 - DNA, 57 bp, synthetic construct
  source 1..57: mol_type = other DNA; note = PC-3
tgccactacagctggttcggtttggtgacttcgttcttcgttgtggtgcttagtggc

SEQ ID NO: 227 - RNA, 15 nt, synthetic construct
  source 1..15: mol_type = other RNA; note = A15
ccctcctacataggg

SEQ ID NO: 228 - RNA, 26 nt, synthetic construct
  source 1..26: mol_type = other RNA; note = AS1411
ggtggtggtggttgtggtggtggtgg

SEQ ID NO: 229 - DNA, 68 bp, synthetic construct
  source 1..68: mol_type = other DNA; note = AS1411
  misc_feature 1..48: note = RNA
  misc_feature 49..68: note = DNA
attctgaaccgtgtgcagcaccacgctgcacacggttcagaatacacacgaggctatctagaatgtac

SEQ ID NO: 230 - RNA, 50 nt, synthetic construct
  source 1..50: mol_type = other RNA; note = BCMA
agtgcaagacgttcgcagattagcgaaaagagggtctcattgactagtac

SEQ ID NO: 231 - RNA, 31 nt, synthetic construct
  source 1..31: mol_type = other RNA; note = CTLA-4
ggtggaagagggatgggccgacgtgccgcat

SEQ ID NO: 232 - DNA, 62 bp, synthetic construct
  source 1..62: mol_type = other DNA; note = CTLA-4
tccctacggcgctaacgatggtgaaaatgggcctagggtggacggtgccaccgtgctacaac

SEQ ID NO: 233 - RNA, 38 nt, synthetic construct
  source 1..38: mol_type = other RNA; note = CCL1
tgactcctctgacagcctaatttctcccgattaccctg

SEQ ID NO: 234 - RNA, 40 nt, synthetic construct
  source 1..40: mol_type = other RNA; note = CEA
ctaggatccccactcaccatctctcagcttgcttcctagc

SEQ ID NO: 235 - RNA, 51 nt, synthetic construct
  source 1..51: mol_type = other RNA; note = CD4-3
gggaggacgatgcggtttggggttttcccgtgccccagacgactcgcccga

SEQ ID NO: 236 - RNA, 102 nt, synthetic construct
  source 1..102: mol_type = other RNA; note = CD28
gggagagaggaagagggatggggattagaccataggctcccaaccccccccgggagagaggaagagggatggggattagaccataggctcccaacccccggg

SEQ ID NO: 237 - RNA, 90 nt, synthetic construct
  source 1..90: mol_type = other RNA; note = CD44
gggatggatccaagcttactggcatctggatttgcgcgtgccagaataaagagtataacgtgtgaatgggaagcttcgataggaattcgg

SEQ ID NO: 238 - DNA, 38 bp, synthetic construct
  source 1..38: mol_type = other DNA; note = PD-L1
ctacgagacgaacttatgcgtaataatgactgtcgtag

SEQ ID NO: 239 - RNA, 39 nt, synthetic construct
  source 1..39: mol_type = other RNA; note = EGFR
gccttagtaacgtgctttgatgtcgattcgacaggaggc

SEQ ID NO: 240 - RNA, 53 nt, synthetic construct
  source 1..53: mol_type = other RNA; note = EGFR
tgccgctataatgcacggatttaatcgccgtagaaaagcatgtcaaagccgtt

SEQ ID NO: 241 - RNA, 19 nt, synthetic construct
  source 1..19: mol_type = other RNA; note = EpCAM
gcgactggttacccggtcg

SEQ ID NO: 242 - RNA, 36 nt, synthetic construct
  source 1..36: mol_type = other RNA; note = FGF2(F2)
gggatactagggcattaatgttaccagtgtagtccc

SEQ ID NO: 243 - RNA, 37 nt, synthetic construct
  source 1..37: mol_type = other RNA; note = FGF2
gggaaactagggcgttaacgtgaccagtgtttctcga

SEQ ID NO: 244 - RNA, 35 nt, synthetic construct
  source 1..35: mol_type = other RNA; note = FGF2
gggaaactagggcgttaacgtgaccagtgtttccc

SEQ ID NO: 245 - RNA, 56 nt, synthetic construct
  source 1..56: mol_type = other RNA; note = FGF5
gggcgacctctccgtactgacctacagagcgacatactagtgtatccagatcgccc

SEQ ID NO: 246 - RNA, 34 nt, synthetic construct
  source 1..34: mol_type = other RNA; note = Her2
agccgcgaggggagggatagggtagggcgcggct

SEQ ID NO: 247 - RNA, 49 nt, synthetic construct
  source 1..49: mol_type = other RNA; note = Her3
cagcgaaagttgcgtatgggtcacatcgcaggcacatgtcatctgggcg

SEQ ID NO: 248 - RNA, 79 nt, synthetic construct
  source 1..79: mol_type = other RNA; note = Her3
gaattccgcgtgtgccagcgaaagttgcgtatgggccacatcgcaggcacatgtcatctgggcggtccgttcgggatcc

SEQ ID NO: 249 - RNA, 70 nt, synthetic construct
  source 1..70: mol_type = other RNA; note = LAG-3
gggagagagatataagggcctcctgatacccgctgctatctggaccgatcccattaccaaattctctccc

SEQ ID NO: 250 - RNA, 25 nt, synthetic construct
  source 1..25: mol_type = other RNA; note = MUC1
gcagttgatcctttggataccctgg

SEQ ID NO: 251 - RNA, 50 nt, synthetic construct
  source 1..50: mol_type = other RNA; note = MRP1
gggagaatagtcaacaaatcgtttggggcgacttctccttcctttctccc

SEQ ID NO: 252 - RNA, 80 nt, synthetic construct
  source 1..80: mol_type = other RNA; note = OX40
gggaggacgatgcggcagtctgcatcgtaggaatcgccaccgtatactttcccaccagacgactcgctgaggatccgaga

SEQ ID NO: 253 - RNA, 69 nt, synthetic construct
  source 1..69: mol_type = other RNA; note = OX40
gggaggacgatgcggcagtctgcatcgtaggaatcgccaccgtatactttcccaccagacgactcgctg

SEQ ID NO: 254 - RNA, 40 nt, synthetic construct
  source 1..40: mol_type = other RNA; note = OX40
cagtctgcatcgtaggaatcgccaccgtatactttcccac

SEQ ID NO: 255 - RNA, 54 nt, synthetic construct
  source 1..54: mol_type = other RNA; note = OX40
gggatgcggaaaaaagaacacttccgattagggcccaccctaacggccgcagac

SEQ ID NO: 256 - RNA, 43 nt, synthetic construct
  source 1..43: mol_type = other RNA; note = PSMA
gggaccgaaaaagacctgacttctatactaagtctacgttccc

SEQ ID NO: 257 - RNA, 39 nt, synthetic construct
  source 1..39: mol_type = other RNA; note = PSMA
gggaggacgatgcggatcagccatgtttacgtcactcct

SEQ ID NO: 258 - RNA, 33 nt, synthetic construct
  source 1..33: mol_type = other RNA; note = PDGFRbeta
tgtcgtggggcatcgagtaaatgcaattcgaca

SEQ ID NO: 259 - RNA, 14 nt, synthetic construct
  source 1..14: mol_type = other RNA; note = TfRA4
gcgtggtaccacgc

SEQ ID NO: 260 - RNA, 14 nt, synthetic construct
  source 1..14: mol_type = other RNA; note = TfRA3
gcgtggtcacacgc

SEQ ID NO: 261 - DNA, 34 bp, synthetic construct; identical to SEQ ID NO: 206
  misc_feature 13..14: note = DNA
  source 1..34: mol_type = other DNA
  misc_feature 1..12: note = RNA
  misc_feature 15..34: note = RNA

SEQ ID NO: 262 - RNA, 61 nt, synthetic construct
  source 1..61: mol_type = other RNA; note = TIM3
gggagaggaccagtagccactatggtgttggagctagcggcagagcgtcgcggtccctccc

SEQ ID NO: 263 - RNA, 61 nt, synthetic construct
  source 1..61: mol_type = other RNA; note = TIM3
gggagaggaccagtactggtagttctctgtgcgactcctacagagcgtcgcggtccctccc

SEQ ID NO: 264 - RNA, 38 nt, synthetic construct
  source 1..38: mol_type = other RNA; note = TIMC-11
aagcaacacttagtcgcgattgatacgtgcgcagtcat

SEQ ID NO: 265 - RNA, 79 nt, synthetic construct
  source 1..79: mol_type = other RNA; note = TIMC-11
ggaggacgatgcggggaagcaacacttagtcgcgattgatacgtgcgcagtcatcagacgactcgctgaggatccgaga

SEQ ID NO: 266 - RNA, 23 nt, synthetic construct
  source 1..23: mol_type = other RNA; note = VEGF
atgcagtttgagaagtcgcgcat

SEQ ID NO: 267 - RNA, 27 nt, synthetic construct
  source 1..27: mol_type = other RNA; note = VEGF165
cggaatcagtgaatgcttatacatccg

SEQ ID NO: 268 - RNA, 96 nt, synthetic construct
  source 1..96: mol_type = other RNA; note = 4-1BB
gggagagaggaagagggatgggcgaccgaacgtgcccttcaaagccgttcactaaccagtggcataacccagaggtcgatagtactggatcccccc

SEQ ID NO: 269 - DNA, 24 bp, synthetic construct
  source 1..24: mol_type = other DNA; note = CPG2006
tcgtcgttttgtcgttttgtcgtt

SEQ ID NO: 270 - RNA, 24 nt, synthetic construct
  source 1..24: mol_type = other RNA; note = CPG2006
tcgtcgttttgtcgttttgtcgtt

SEQ ID NO: 271 - DNA, 18 bp, synthetic construct
  source 1..18: mol_type = other DNA; note = CPG1826
tccatgacgttcctgacg

SEQ ID NO: 272 - DNA, 20 bp, synthetic construct
  source 1..20: mol_type = other DNA; note = CPG2216
gggggacgatcgtcgggggg

SEQ ID NO: 273 - DNA, 22 bp, synthetic construct
  source 1..22: mol_type = other DNA; note = CPG2395
tcgtcgttttcggcgcgcgccg

SEQ ID NO: 274 - DNA, 21 bp, synthetic construct
  source 1..21: mol_type = other DNA; note = CPG-ODNT7
tcgtcgtcgtcgtcgtcgtcg

SEQ ID NO: 275 - DNA, 24 bp, synthetic construct
  source 1..24: mol_type = other DNA; note = CPG-ODNT7
tcgtcgtcgtcgtcgtcgtcgtcg

SEQ ID NO: 276 - DNA, 16 bp, synthetic construct
  source 1..16: mol_type = other DNA; note = transition base segment
ttgcggcgagcggcga

SEQ ID NO: 277 - DNA, 16 bp, synthetic construct
  source 1..16: mol_type = other DNA; note = complementary sequence
tcgccgctcgccgctt

SEQ ID NO: 278 - DNA, 14 bp, synthetic construct
  source 1..14: mol_type = other DNA; note = d sequence
gccaccgtgctaca

SEQ ID NO: 279 - DNA, 14 bp, synthetic construct
  source 1..14: mol_type = other DNA; note = e sequence
cagcagcagcagca

SEQ ID NO: 280 - DNA, 13 bp, synthetic construct
  source 1..13: mol_type = other DNA; note = transition base segment
gtagcacggtggc

SEQ ID NO: 281 - DNA, 68 bp, synthetic construct
  source 1..68: mol_type = other DNA; note = B sequence
gccttagtaacgtgctttgatgtcgattcgacaggaggctttttgctcccggttcgccgccagccgcc

SEQ ID NO: 282 - DNA, 57 bp, synthetic construct
  source 1..57: mol_type = other DNA; note = A sequence
ggtggtggtggttgtggtggtggtggtttttgcggcgcccacgagcgttccgggagc

SEQ ID NO: 283 - DNA, 68 bp, synthetic construct; identical to SEQ ID NO: 281
  source 1..68: mol_type = other DNA; note = B sequence

SEQ ID NO: 284 - DNA, 51 bp, synthetic construct
  source 1..51: mol_type = other DNA; note = C sequence
ccctcctacatagggtttttggcggcaggcggccatagccgtgggcgccgc

SEQ ID NO: 285 - DNA, 55 bp, synthetic construct
  source 1..55: mol_type = other DNA; note = B sequence
ggtggtggtggttgtggtggtggtggtttttgctcccggttcgccgccagccgcc

SEQ ID NO: 286 - DNA, 33 bp, synthetic construct
  source 1..33: mol_type = other DNA; note = TTA1
ctgcacttggcttggatttcagaagggagaccc

SEQ ID NO: 287 - DNA, 74 bp, synthetic construct
  source 1..74: mol_type = other DNA; note = B sequence
ggttgcatgccgtggggaggggggtgggttttatagcgtactcagtttttgctcccggttcgccgccagccgcc

SEQ ID NO: 288 - DNA, 51 bp, synthetic construct; identical to SEQ ID NO: 284
  source 1..51: mol_type = other DNA; note = C sequence

SEQ ID NO: 289 - DNA, 57 bp, synthetic construct; identical to SEQ ID NO: 282
  source 1..57: mol_type = other DNA; note = A sequence

SEQ ID NO: 290 - DNA, 68 bp, synthetic construct; identical to SEQ ID NO: 281
  source 1..68: mol_type = other DNA; note = B sequence

SEQ ID NO: 291 - DNA, 59 bp, synthetic construct
  source 1..59: mol_type = other DNA; note = C sequence
ccctcctacatagggtttttggcggcaggcggccatagccgtgggcgccgcgataagct

SEQ ID NO: 292 - DNA, 57 bp, synthetic construct
  source 1..57: mol_type = other DNA; note = A sequence
gcgtggtaccacgctttttgcggcgagcggcgcccacgagcgttccgggagaggagc

SEQ ID NO: 293 - DNA, 60 bp, synthetic construct
  source 1..60: mol_type = other DNA; note = B sequence
ggtggtggtggttgtggtggtggtggtttttgctcctctcccggttcgccgccagccgcc

SEQ ID NO: 294 - DNA, 58 bp, synthetic construct
  source 1..58: mol_type = other DNA; note = C sequence
ccctcctacatagggtttttggcggctggcggccatagccgtgggcgccgctcgccgc

SEQ ID NO: 295 - DNA, 67 bp, synthetic construct
  source 1..67: mol_type = other DNA; note = A sequence
tcgccgctcgccgcttgcgtggtaccacgcttgcggcgagcggcgagcccacgagcgttccgggaga

SEQ ID NO: 296 - DNA, 55 bp, synthetic construct
  source 1..55: mol_type = other DNA; note = B sequence
ggtggtggtggttgtggtggtggtggttttttctcccggttcgccgccagccgcc

SEQ ID NO: 297 - DNA, 46 bp, synthetic construct
  source 1..46: mol_type = other DNA; note = C sequence
ccctcctacatagggtttttggcggctggcggccatagccgtgggc

SEQ ID NO: 298 - DNA, 57 bp, synthetic construct; identical to SEQ ID NO: 282
  source 1..57: mol_type = other DNA; note = A sequence

SEQ ID NO: 299 - DNA, 43 bp, synthetic construct
  source 1..43: mol_type = other DNA; note = B sequence
gcgtggtcacacgctttttgctcccggttcgccgccagccgcc

SEQ ID NO: 300 - DNA, 51 bp, synthetic construct; identical to SEQ ID NO: 284
  source 1..51: mol_type = other DNA; note = C sequence

SEQ ID NO: 301 - DNA, 60 bp, synthetic construct
  source 1..60: mol_type = other DNA; note = A sequence
tcgtcgttttgtcgttttgtcgtttttttgcgacgcccacgagcgttccgggagaggagc

SEQ ID NO: 302 - DNA, 59 bp, synthetic construct
  source 1..59: mol_type = other DNA; note = B sequence
ccaacgagtaggcgatagcgcgtggtttttgctcctctcccggttcgccgcgagccgcg

SEQ ID NO: 303 - DNA, 81 bp, synthetic construct
  source 1..81: mol_type = other DNA; note = C sequence
acgggccacatcaactcattgatagacaatgcgtccactgcccgttttttcgcggctcgcggccatagccgtgggcgtcgc

SEQ ID NO: 304 - DNA, 55 bp, synthetic construct
  source 1..55: mol_type = other DNA; note = A sequence
tcgtcgttttgtcgttttgtcgtttttttgacgcccacgagcgttccgggagagg

SEQ ID NO: 305 - DNA, 67 bp, synthetic construct
  source 1..67: mol_type = other DNA; note = B sequence
ccaacgagtaggcgatagcgcgtggtttttcctctcccggttcgccgcgagcctgtagcacggtggc

SEQ ID NO: 306 - DNA, 68 bp, synthetic construct
  source 1..68: mol_type = other DNA; note = C sequence
tcgtcgttttgtcgttttgtcgttttttggctcgcggccatagccgtgggcgtctgctgctgctgctg

SEQ ID NO: 307 - DNA, 64 bp, synthetic construct
  source 1..64: mol_type = other DNA; note = D sequence
acgggccacatcaactcattgatagacaatgcgtccactgcccgttttttgccaccgtgctaca

SEQ ID NO: 308 - DNA, 54 bp, synthetic construct
  source 1..54: mol_type = other DNA; note = E sequence
gtggattgttgtgttctgttggtttttgtgttgtctttttcagcagcagcagca

SEQ ID NO: 309 - DNA, 60 bp, synthetic construct; identical to SEQ ID NO: 301
  source 1..60: mol_type = other DNA; note = A sequence

SEQ ID NO: 310 - DNA, 50 bp, synthetic construct
  source 1..50: mol_type = other DNA; note = B sequence
  misc_feature 1..21: note = RNA
  misc_feature 22..50: note = DNA
ggtgattacccagagatatttgctcctctcccggttcgccgcgagccgcg

SEQ ID NO: 311 - DNA, 52 bp, synthetic construct
  source 1..52: mol_type = other DNA; note = C sequence
  misc_feature 1..21: note = RNA
  misc_feature 22..52: note = DNA
ccagcacactgagaatcaattcgcggctcgcggccatagccgtgggcgtcgc

SEQ ID NO: 312 - DNA, 61 bp, synthetic construct
  source 1..61: mol_type = other DNA; note = D sequence
  misc_feature 1..40: note = DNA
  misc_feature 41..61: note = RNA
gtggattgttgtgttctgttggtttttgtgttgtctttttatatctctgggtaatcacctt

SEQ ID NO: 313 - DNA, 59 bp, synthetic construct
  source 1..59: mol_type = other DNA; note = E sequence
  misc_feature 1..38: note = DNA
  misc_feature 39..59: note = RNA
gccccagttatgctttccccctctgtctctttgtttttttgattctcagtgtgctggtt

SEQ ID NO: 314 - DNA, 45 bp, synthetic construct
  source 1..45: mol_type = other DNA; note = A sequence
gcgtggtaccacgctttttgcggcgcccacgagcgttccgggagc

SEQ ID NO: 315 - DNA, 79 bp, synthetic construct
  source 1..79: mol_type = other DNA; note = B sequence
acgggccacatcaactcattgatagacaatgcgtccactgcccgttttttgctcctctcccggttcgccgcgagccgcg

SEQ ID NO: 316 - DNA, 54 bp, synthetic construct
  source 1..54: mol_type = other DNA; note = C sequence
  misc_feature 1..33: note = DNA
  misc_feature 34..52: note = RNA
  misc_feature 53..54: note = DNA
cgcggctcgcggccatagccgtgggcgtcgcaatcatagatggcgttgttgctt

SEQ ID NO: 317 - DNA, 39 bp, synthetic construct
  source 1..39: mol_type = other DNA; note = D sequence
  misc_feature 1..18: note = DNA
  misc_feature 19..37: note = RNA
  misc_feature 38..39: note = DNA
gataagctgataagctaagcaacaacgccatctatgatt

SEQ ID NO: 318 - DNA, 72 bp, synthetic construct
  source 1..72: mol_type = other DNA; note = A sequence
  misc_feature 1..50: note = DNA
  misc_feature 51..72: note = RNA
gcgtggtaccacgctttttgcggcgcccacgagcgttccgggagaggagctttgattctcagtgtgctggtt

SEQ ID NO: 319 - DNA, 51 bp, synthetic construct
  source 1..51: mol_type = other DNA; note = B sequence
  misc_feature 1..21: note = RNA
  misc_feature 22..51: note = DNA
ccagcacactgagaatcaattgctcctctcccggttcgccgccagccgcgg

SEQ ID NO: 320 - DNA, 79 bp, synthetic construct
  source 1..79: mol_type = other DNA; note = C sequence
  misc_feature 1..57: note = DNA
  misc_feature 58..79: note = RNA
aacggagtgtggctaactcgatttttggcggctggcggccatagccgtgggcgccgctggtgattacccagagatattt

SEQ ID NO: 321 - DNA, 64 bp, synthetic construct
  source 1..64: mol_type = other DNA; note = D sequence
  misc_feature 1..40: note = RNA
  misc_feature 41..43: note = DNA
  misc_feature 44..64: note = RNA
aaaaagcaacagggtgctccatgcgcatggaacctgcgcgaaaatatctctgggtaatcacctt

SEQ ID NO: 322 - DNA, 68 bp, synthetic construct
  source 1..68: mol_type = other DNA; note = A sequence
  modified_base 27..32: mod_base = OTHER; note = 5-fluorouracil (5-FU)
  modified_base 63..68: mod_base = OTHER; note = 5-fluorouracil (5-FU)
  misc_feature 1..26: note = DNA
  misc_feature 27..68: note = RNA
ggtggtggtggttgtggtggtggtggnnnnnngcggcgcccacgagcgttccgggagaggccnnnnnn

SEQ ID NO: 323 - RNA, 79 nt, synthetic construct
  source 1..79: mol_type = other RNA; note = B sequence
  modified_base 40..45: mod_base = OTHER; note = 5-fluorouracil (5-FU)
  modified_base 74..79: mod_base = OTHER; note = 5-fluorouracil (5-FU)
gccttagtaacgtgctttgatgtcgattcgacaggaggcnnnnnnggcctctcccggttcgccgccagccgccnnnnnn

SEQ ID NO: 324 - RNA, 58 nt, synthetic construct
  source 1..58: mol_type = other RNA; note = C sequence
  modified_base 53..58: mod_base = OTHER; note = 5-fluorouracil (5-FU)
  modified_base 16..21: mod_base = OTHER; note = 5-fluorouracil (5-FU)
ccctcctacatagggnnnnnnggcggctggcggccatagccgtgggcgccgcnnnnnn

SEQ ID NO: 325 - DNA, 64 bp, synthetic construct
  source 1..64: mol_type = other DNA; note = A sequence
ggtggtggtggttgtggtggtggtggtttttgcggcgcccacgagcgttccgggagaggaggcc

SEQ ID NO: 326 - DNA, 75 bp, synthetic construct
  source 1..75: mol_type = other DNA; note = B sequence
gccttagtaacgtgctttgatgtcgattcgacaggaggctttttggcctcctctcccggttcgccgccagccgcc

SEQ ID NO: 327 - DNA, 51 bp, synthetic construct; identical to SEQ ID NO: 68
  source 1..51: mol_type = other DNA; note = C sequence

SEQ ID NO: 328 - DNA, 62 bp, synthetic construct
  source 1..62: mol_type = other DNA; note = A sequence
ggtggtggtggttgtggtggtggtggtttttgcggcgcccacgagcgttccgggagaggagc